European Patent Specification EP 4 182 480 B1, published May 7, 2025. Title: PROGNOSTIC BIOMARKERS FOR CANCER. Applicant: European Molecular Biology Laboratory. The sequence listing filed with the application follows.

SEQUENCE LISTING (19 sequences)

SEQ ID NO: 1 - RNA, 5 nt, Homo sapiens
agacu

SEQ ID NO: 2 - RNA, 5 nt, Homo sapiens
ggacu

SEQ ID NO: 3 - RNA, 5 nt, Homo sapiens
ugacu

SEQ ID NO: 4 - RNA, 5 nt, Homo sapiens
aaacu

SEQ ID NO: 5 - RNA, 5 nt, Homo sapiens
gaacu

SEQ ID NO: 6 - RNA, 5 nt, Homo sapiens
uaacu

SEQ ID NO: 7 - RNA, 5 nt, Homo sapiens
agaca

SEQ ID NO: 8 - RNA, 5 nt, Homo sapiens
ggaca

SEQ ID NO: 9 - RNA, 5 nt, Homo sapiens
ugaca

SEQ ID NO: 10 - RNA, 5 nt, Homo sapiens
aaaca

SEQ ID NO: 11 - RNA, 5 nt, Homo sapiens
gaaca

SEQ ID NO: 12 - RNA, 5 nt, Homo sapiens
uaaca

SEQ ID NO: 13 - RNA, 5 nt, Homo sapiens
agacc

SEQ ID NO: 14 - RNA, 5 nt, Homo sapiens
ggacc

SEQ ID NO: 15 - RNA, 5 nt, Homo sapiens
ugacc

SEQ ID NO: 16 - RNA, 5 nt, Homo sapiens
aaacc

SEQ ID NO: 17 - RNA, 5 nt, Homo sapiens
gaacc

SEQ ID NO: 18 - RNA, 5 nt, Homo sapiens
uaacc

SEQ ID NO: 19 - RNA, 9 nt, Homo sapiens
aggagacug